European Patent Application EP 4 484 418 A1, published January 1, 2025. Title: USE OF NOVEL POMALIDOMIDE DERIVATIVE FOR TREATING BRAIN DISEASE. Applicant: Aevis Bio, Inc. The sequence listing filed with the application follows.

SEQUENCE LISTING (6 sequences)

SEQ ID NO: 1 - DNA, 20 bp, synthetic construct
  source 1..20: mol_type = other DNA
gctatggccgctttgatgtg

SEQ ID NO: 2 - DNA, 20 bp, synthetic construct
  source 1..20: mol_type = other DNA
ttgggatgctccatggtcac

SEQ ID NO: 3 - DNA, 25 bp, synthetic construct
  source 1..25: mol_type = other DNA
ctggaacatggactcactcagtttg

SEQ ID NO: 4 - DNA, 20 bp, synthetic construct
  source 1..20: mol_type = other DNA
aggcctttgccactgcttgt

SEQ ID NO: 5 - DNA, 24 bp, synthetic construct
  source 1..24: mol_type = other DNA
ttcaacagcaactcccactcttcc

SEQ ID NO: 6 - DNA, 23 bp, synthetic construct
  source 1..23: mol_type = other DNA
tggtccagggtttcttactcctt